European Patent Application EP 4 296 669 A1, published December 27, 2023. Title: High-throughput screening for ligands of transmembrane proteins. Applicant: LenioBio GmbH. The sequence listing filed with the application follows.

SEQUENCE LISTING (33 sequences)

SEQ ID NO: 1 - DNA, 21 bp, Artificial Sequence
  Primer P0001
gtacgcaccacgtgtgattac

SEQ ID NO: 2 - DNA, 26 bp, Artificial Sequence
  Primer P0002
tcacatgtaatacgactcactatagg

SEQ ID NO: 3 - DNA, 31 bp, Artificial Sequence
  Primer P0750
tagtaataaggatcctctagaggtaccaagc

SEQ ID NO: 4 - DNA, 19 bp, Artificial Sequence
  Primer P0751
catggcagccgcatagatg

SEQ ID NO: 5 - DNA, 23 bp, Artificial Sequence
  Primer P0752
catggcagccgcatagatgtaag

SEQ ID NO: 6 - DNA, 48 bp, Artificial Sequence
  Primer P0753
tctatgcggctgccatggctccgtcatcaacaagtttgtacaaaaaag

SEQ ID NO: 7 - DNA, 45 bp, Artificial Sequence
  Primer P0754
tctatgcggctgccatggctccgtcatcaacaagtttgtacaaaa

SEQ ID NO: 8 - DNA, 43 bp, Artificial Sequence
  Primer P0755
cctctagaggatccttattactattttggaggatggtcgccac

SEQ ID NO: 9 - DNA, 31 bp, Artificial Sequence; identical to SEQ ID NO: 3
  Primer P0756

SEQ ID NO: 10 - DNA, 19 bp, Artificial Sequence
  Primer P0757
catggcagccgcatagatg

SEQ ID NO: 11 - DNA, 41 bp, Artificial Sequence
  Primer P0758
tctatgcggctgccatggctatggcagaaatcggtactggc

SEQ ID NO: 12 - DNA, 48 bp, Artificial Sequence
  Primer P0759
cctctagaggatccttattactataccactttgtacaagaaagctggg

SEQ ID NO: 13 - DNA, 77 bp, Artificial Sequence
  Primer P0760
gtacctctagaggatccttattactatttctcgaactgtggatgggaccatgcaaccactttgtacaagaaagctgg

SEQ ID NO: 14 - DNA, 35 bp, Artificial Sequence
  Primer P0761
tatgcggctgccatggctgctccgtcatcaacaag

SEQ ID NO: 15 - DNA, 28 bp, Artificial Sequence
  Primer P0762
taataaggatcctctagaggtaccaagc

SEQ ID NO: 16 - DNA, 34 bp, Artificial Sequence
  Primer P0763
catggcagccgcatagatgtaagaaatgtatacg

SEQ ID NO: 17 - DNA, 39 bp, Artificial Sequence
  Primer P0764
aaaagcgctgaaaacctggctccgtcatcaacaagtttg

SEQ ID NO: 18 - DNA, 48 bp, Artificial Sequence
  Primer P0765
cctctagaggatccttattactaaaccactttgtacaagaaagctggg

SEQ ID NO: 19 - DNA, 31 bp, Artificial Sequence; identical to SEQ ID NO: 3
  Primer P0766

SEQ ID NO: 20 - DNA, 24 bp, Artificial Sequence
  Primer P0767
caggttttcagcgcttttttcgaa

SEQ ID NO: 21 - DNA, 23 bp, Artificial Sequence
  Primer P0768
ctctgcacgctcttttggacaac

SEQ ID NO: 22 - DNA, 22 bp, Artificial Sequence
  Primer P0769
gcatttatggagttcatccgcc

SEQ ID NO: 23 - DNA, 44 bp, Artificial Sequence
  Primer P0770
gtatacatttcttacatctatgcgatgtcaagctcttcctggct

SEQ ID NO: 24 - DNA, 37 bp, Artificial Sequence
  Primer P0771
tggatgggaccatgccaaaaaggaggtctgaacatca

SEQ ID NO: 25 - DNA, 19 bp, Artificial Sequence
  Primer P0772
gcatggtcccatccacagt

SEQ ID NO: 26 - DNA, 40 bp, Artificial Sequence
  Primer P0773
gtatacatttcttacatctatgcgatggcccgagccatgg

SEQ ID NO: 27 - DNA, 30 bp, Artificial Sequence
  Primer P0774
tggatgggaccatgcccttgtgccctctgt

SEQ ID NO: 28 - DNA, 41 bp, Artificial Sequence
  Primer P0775
gtatacatttcttacatctatgcgatgcgctggtgtctcct

SEQ ID NO: 29 - DNA, 34 bp, Artificial Sequence
  Primer P0776
tggatgggaccatgcaccagtctctgtgaagaag

SEQ ID NO: 30 - DNA, 35 bp, Artificial Sequence
  Primer P0777
tggatgggaccatgcttttggaggatggtcgccac

SEQ ID NO: 31 - DNA, 45 bp, Artificial Sequence
  Primer P0778
gtatacatttcttacatctatgcgaatgtcaagctcttcctggct

SEQ ID NO: 32 - DNA, 40 bp, Artificial Sequence; identical to SEQ ID NO: 26
  Primer P0779

SEQ ID NO: 33 - DNA, 42 bp, Artificial Sequence
  Primer P0780
gtatacatttcttacatctatgcgaatgcgctggtgtctcct